European Patent Application EP 4 613 768 A1, published September 10, 2025. Title: GIPR binding protein and use thereof. Applicant: Suzhou Alphamab Co., Ltd. Application EP. The sequence listing filed with the application follows.

SEQUENCE LISTING (113 sequences)

SEQ ID NO: 1 - protein, 115 aa, synthetic construct
QVQLVESGGGLVQPGGSLRLSCETSKILFSSAYTMGWYRQAPGKQRELVATITTDYITNYVDSVKGRFTISRDNAKNTVYLQMNTLKLEDTAVYYCNARWGRDYWGQGTQVTVSS

SEQ ID NO: 2 - protein, 121 aa, synthetic construct
QVQLVESGGALVQTGGSLRLFCAASGDTICITNMNWYRQAPGKGREFVAAITRSGRTLYADYVKGRFTISRDNARNTMSLQMNSMTSEDTAVYYCNADQNQTICAAEPSAWGRGTQVTVSS

SEQ ID NO: 3 - protein, 123 aa, synthetic construct
QVQLVESGGGLVQAGGSLKLSCAASGRTFSSKAMGWFRQAPGKEREFVAAINWSGDRTYHVNSIKGRFTISRDNAKNTVYLQMNSLKPEDTAVYYCTADRRDRATIPFQWHYWGQGTQVTVSS

SEQ ID NO: 4 - protein, 122 aa, synthetic construct
QVQLVESGGKLVQAGGSLRLDCVASGRTFSYYAIGWYRQAPGKEREFVAAIRASGGSTYYADSVKGRFTASRDNAKNTGYLQMNSLKPEDTAVYFCYAATIVPITPSTHGYWGQGTQVTVSS

SEQ ID NO: 5 - protein, 130 aa, synthetic construct
QVQLVESGGGLVQPGGSLRLSCAASRYTLDYYAIGWFRQAPGKEREGVSCINSKDGSTYYADSVKGRFTISKDNAKNTVYLQMNSLKPEDTAVYYCAAGYDPWSGIPPVQAMCVMGYDYWGQGTQVTVSS

SEQ ID NO: 6 - protein, 122 aa, synthetic construct
QVQLQESGGGLVQPGGSLRLSCVASGSGFSIVAMGWYRQTPGKQRELVAAITSGGNTNYADSVKGRFTISRDNAKNTIYLQMNSLKPEDTAVYYCNADPGVVAGPYAGMDFWGKGTQVTVSS

SEQ ID NO: 7 - protein, 110 aa, synthetic construct
QVQLQESGGSLRLSCAASGPIFSFTTMAWYRQVPGKQRELVASITTGGSTAYTDSVKGRFTISRDNAKSTLYLQMNNLKPEDTAVYYCNTGPRNVWAAAWGQGTQVTVSS

SEQ ID NO: 8 - protein, 130 aa, synthetic construct
EVQLVESGGGLVQPGGSLRLSCAASRYTLDYYAIGWFRQAPGKEREGVSCINSKDGSTYYADSVKGRFTISKDNSKNTVYLQMNSLRAEDTAVYYCAAGYDPWSGIPPVQAMCVMGYDYWGQGTLVTVSS

SEQ ID NO: 9 - protein, 130 aa, synthetic construct
EVQLVESGGGLVQPGGSLRLSCAASRYTLDYYAIGWFRQAPGKEREGVSCINSKDGSTYYADSVKGRFTISRDNSKNTVYLQMNSLRAEDTAVYYCAAGYDPWSGIPPVQAMCVMGYDYWGQGTLVTVSS

SEQ ID NO: 10 - protein, 130 aa, synthetic construct
EVQLVESGGGLVQPGGSLRLSCAASRYTLDYYAIGWFRQAPGKGLEGVSCINSKDGSTYYADSVKGRFTISKDNSKNTVYLQMNSLRAEDTAVYYCAAGYDPWSGIPPVQAMCVMGYDYWGQGTLVTVSS

SEQ ID NO: 11 - protein, 130 aa, synthetic construct
EVQLVESGGGLVQPGGSLRLSCAASRYTLDYYAIGWFRQAPGKGLEGVSCINSKDGSTYYADSVKGRFTISRDNSKNTVYLQMNSLRAEDTAVYYCAAGYDPWSGIPPVQAMCVMGYDYWGQGTLVTVSS

SEQ ID NO: 12 - protein, 130 aa, synthetic construct
QVQLVESGGGLVQPGGSLRLSCSASRYTLDYYAIGWFRQAPGKEREGVSCINSKDGSTYYADSVKGRFTISKDNSKNTVYLQMNSLRAEDTAVYYCAAGYDPWSGIPPVQAMCVMGYDYWGQGTLVTVSS

SEQ ID NO: 13 - protein, 130 aa, synthetic construct
QVQLVESGGGLVQPGGSLRLSCSASRYTLDYYAIGWFRQAPGKEREGVSCINSKDGSTYYADSVKGRFTISRDNSKNTVYLQMNSLRAEDTAVYYCAAGYDPWSGIPPVQAMCVMGYDYWGQGTLVTVSS

SEQ ID NO: 14 - protein, 130 aa, synthetic construct
QVQLVESGGGLVQPGGSLRLSCSASRYTLDYYAIGWFRQAPGKGLEGVSCINSKDGSTYYADSVKGRFTISKDNSKNTVYLQMNSLRAEDTAVYYCAAGYDPWSGIPPVQAMCVMGYDYWGQGTLVTVSS

SEQ ID NO: 15 - protein, 122 aa, synthetic construct
QVQLVESGGGLVQPGGSLRLSCSASGSGFSIVAMGWVRQAPGKGLELVAAITSGGNTNYADSVKGRFTISRDNSKNTIYLQMNSLRAEDTAVYYCNADPGVVAGPYAGMDFWGKGTTVTVSS

SEQ ID NO: 16 - protein, 122 aa, synthetic construct
QVQLQESGGGLVQPGGSLRLSCSASGSGFSIVAMGWVRQTPGKGLELVAAITSGGNTNYADSVKGRFTISRDNSKNTIYLQMNSLRAEDTAVYYCNADPGVVAGPYAGMDFWGKGTTVTVSS

SEQ ID NO: 17 - protein, 122 aa, synthetic construct
QVQLQESGGGLVQPGGSLRLSCSASGSGFSIVAMGWVRQTPGKGLELVAAITSGGNTNYADSVKGRFTISRDNAKNTIYLQMNSLRAEDTAVYYCNADPGVVAGPYAGMDFWGKGTTVTVSS

SEQ ID NO: 18 - protein, 122 aa, synthetic construct
QVQLVESGGGLVQPGGSLRLSCSASGSGFSIVAMGWVRQAPGKQRELVAAITSGGNTNYADSVKGRFTISRDNSKNTIYLQMNSLRAEDTAVYYCNADPGVVAGPYAGMDFWGKGTTVTVSS

SEQ ID NO: 19 - protein, 122 aa, synthetic construct
QVQLQESGGGLVQPGGSLRLSCSASGSGFSIVAMGWVRQTPGKQRELVAAITSGGNTNYADSVKGRFTISRDNAKNTIYLQMNSLRAEDTAVYYCNADPGVVAGPYAGMDFWGKGTTVTVSS

SEQ ID NO: 20 - protein, 122 aa, synthetic construct
QVQLQESGGGLVQPGGSLRLSCSASGSGFSIVAMGWVRQTPGKQRELVAAITSGGNTNYADSVKGRFTISRDNAKNTIYLQMNSLKPEDTAVYYCNADPGVVAGPYAGMDFWGKGTTVTVSS

SEQ ID NO: 21 - protein, 122 aa, synthetic construct
QVQLVESGGGLVQPGGSLRLSCSASGSGFSIVAMGWYRQTPGKGLELVAAITSGGNTNYADSVKGRFTISRDNSKNTIYLQMNSLRAEDTAVYYCNADPGVVAGPYAGMDFWGKGTTVTVSS

SEQ ID NO: 22 - protein, 122 aa, synthetic construct
QVQLQESGGGLVQPGGSLRLSCSASGSGFSIVAMGWYRQTPGKGLELVAAITSGGNTNYADSVKGRFTISRDNSKNTIYLQMNSLRAEDTAVYYCNADPGVVAGPYAGMDFWGKGTTVTVSS

SEQ ID NO: 23 - protein, 122 aa, synthetic construct
QVQLVESGGGLVQPGGSLRLSCSASGSGFSIVAMGWYRQTPGKQRELVAAITSGGNTNYADSVKGRFTISRDNSKNTIYLQMNSLRAEDTAVYYCNADPGVVAGPYAGMDFWGKGTTVTVSS

SEQ ID NO: 24 - protein, 122 aa, synthetic construct
QVQLQESGGGLVQPGGSLRLSCSASGSGFSIVAMGWYRQTPGKQRELVAAITSGGNTNYADSVKGRFTISRDNAKNTIYLQMNSLRAEDTAVYYCNADPGVVAGPYAGMDFWGKGTTVTVSS

SEQ ID NO: 25 - protein, 122 aa, synthetic construct
QVQLQESGGGLVQPGGSLRLSCSASGSGFSIVAMGWYRQTPGKQRELVAAITSGGNTNYADSVKGRFTISRDNAKNTIYLQMNSLKPEDTAVYYCNADPGVVAGPYAGMDFWGKGTTVTVSS

SEQ ID NO: 26 - protein, 6 aa, synthetic construct
SAYTMG

SEQ ID NO: 27 - protein, 16 aa, synthetic construct
TITTDYITNYVDSVKG

SEQ ID NO: 28 - protein, 6 aa, synthetic construct
RWGRDY

SEQ ID NO: 29 - protein, 11 aa, synthetic construct
KILFSSAYTMG

SEQ ID NO: 30 - protein, 9 aa, synthetic construct
TITTDYITN

SEQ ID NO: 31 - protein, 6 aa, synthetic construct
RWGRDY

SEQ ID NO: 32 - protein, 8 aa, synthetic construct
KILFSSAY

SEQ ID NO: 33 - protein, 5 aa, synthetic construct
TTDYI

SEQ ID NO: 34 - protein, 6 aa, synthetic construct
RWGRDY

SEQ ID NO: 35 - protein, 9 aa, synthetic construct
KILFSSAYT

SEQ ID NO: 36 - protein, 7 aa, synthetic construct
ITTDYIT

SEQ ID NO: 37 - protein, 8 aa, synthetic construct
NARWGRDY

SEQ ID NO: 38 - protein, 5 aa, synthetic construct
ITNMN

SEQ ID NO: 39 - protein, 16 aa, synthetic construct
AITRSGRTLYADYVKG

SEQ ID NO: 40 - protein, 13 aa, synthetic construct
DQNQTICAAEPSA

SEQ ID NO: 41 - protein, 10 aa, synthetic construct
GDTICITNMN

SEQ ID NO: 42 - protein, 9 aa, synthetic construct
AITRSGRTL

SEQ ID NO: 43 - protein, 13 aa, synthetic construct
DQNQTICAAEPSA

SEQ ID NO: 44 - protein, 7 aa, synthetic construct
GDTICIT

SEQ ID NO: 45 - protein, 5 aa, synthetic construct
TRSGR

SEQ ID NO: 46 - protein, 13 aa, synthetic construct
DQNQTICAAEPSA

SEQ ID NO: 47 - protein, 8 aa, synthetic construct
GDTICITN

SEQ ID NO: 48 - protein, 7 aa, synthetic construct
ITRSGRT

SEQ ID NO: 49 - protein, 15 aa, synthetic construct
NADQNQTICAAEPSA

SEQ ID NO: 50 - protein, 5 aa, synthetic construct
SKAMG

SEQ ID NO: 51 - protein, 17 aa, synthetic construct
AINWSGDRTYHVNSIKG

SEQ ID NO: 52 - protein, 14 aa, synthetic construct
DRRDRATIPFQWHY

SEQ ID NO: 53 - protein, 10 aa, synthetic construct
GRTFSSKAMG

SEQ ID NO: 54 - protein, 10 aa, synthetic construct
AINWSGDRTY

SEQ ID NO: 55 - protein, 14 aa, synthetic construct
DRRDRATIPFQWHY

SEQ ID NO: 56 - protein, 7 aa, synthetic construct
GRTFSSK

SEQ ID NO: 57 - protein, 6 aa, synthetic construct
NWSGDR

SEQ ID NO: 58 - protein, 14 aa, synthetic construct
DRRDRATIPFQWHY

SEQ ID NO: 59 - protein, 8 aa, synthetic construct
GRTFSSKA

SEQ ID NO: 60 - protein, 8 aa, synthetic construct
INWSGDRT

SEQ ID NO: 61 - protein, 16 aa, synthetic construct
TADRRDRATIPFQWHY

SEQ ID NO: 62 - protein, 5 aa, synthetic construct
YYAIG

SEQ ID NO: 63 - protein, 17 aa, synthetic construct
AIRASGGSTYYADSVKG

SEQ ID NO: 64 - protein, 13 aa, synthetic construct
ATIVPITPSTHGY

SEQ ID NO: 65 - protein, 10 aa, synthetic construct
GRTFSYYAIG

SEQ ID NO: 66 - protein, 10 aa, synthetic construct
AIRASGGSTY

SEQ ID NO: 67 - protein, 13 aa, synthetic construct
ATIVPITPSTHGY

SEQ ID NO: 68 - protein, 7 aa, synthetic construct
GRTFSYY

SEQ ID NO: 69 - protein, 6 aa, synthetic construct
RASGGS

SEQ ID NO: 70 - protein, 13 aa, synthetic construct
ATIVPITPSTHGY

SEQ ID NO: 71 - protein, 8 aa, synthetic construct
GRTFSYYA

SEQ ID NO: 72 - protein, 8 aa, synthetic construct
IRASGGST

SEQ ID NO: 73 - protein, 15 aa, synthetic construct
YAATIVPITPSTHGY

SEQ ID NO: 74 - protein, 5 aa, synthetic construct
YYAIG

SEQ ID NO: 75 - protein, 17 aa, synthetic construct
CINSKDGSTYYADSVKG

SEQ ID NO: 76 - protein, 21 aa, synthetic construct
GYDPWSGIPPVQAMCVMGYDY

SEQ ID NO: 77 - protein, 10 aa, synthetic construct
RYTLDYYAIG

SEQ ID NO: 78 - protein, 10 aa, synthetic construct
CINSKDGSTY

SEQ ID NO: 79 - protein, 21 aa, synthetic construct
GYDPWSGIPPVQAMCVMGYDY

SEQ ID NO: 80 - protein, 7 aa, synthetic construct
RYTLDYY

SEQ ID NO: 81 - protein, 6 aa, synthetic construct
NSKDGS

SEQ ID NO: 82 - protein, 21 aa, synthetic construct
GYDPWSGIPPVQAMCVMGYDY

SEQ ID NO: 83 - protein, 8 aa, synthetic construct
RYTLDYYA

SEQ ID NO: 84 - protein, 8 aa, synthetic construct
INSKDGST

SEQ ID NO: 85 - protein, 23 aa, synthetic construct
AAGYDPWSGIPPVQAMCVMGYDY

SEQ ID NO: 86 - protein, 5 aa, synthetic construct
IVAMG

SEQ ID NO: 87 - protein, 16 aa, synthetic construct
AITSGGNTNYADSVKG

SEQ ID NO: 88 - protein, 14 aa, synthetic construct
DPGVVAGPYAGMDF

SEQ ID NO: 89 - protein, 10 aa, synthetic construct
GSGFSIVAMG

SEQ ID NO: 90 - protein, 9 aa, synthetic construct
AITSGGNTN

SEQ ID NO: 91 - protein, 14 aa, synthetic construct
DPGVVAGPYAGMDF

SEQ ID NO: 92 - protein, 7 aa, synthetic construct
GSGFSIV

SEQ ID NO: 93 - protein, 5 aa, synthetic construct
TSGGN

SEQ ID NO: 94 - protein, 14 aa, synthetic construct
DPGVVAGPYAGMDF

SEQ ID NO: 95 - protein, 8 aa, synthetic construct
GSGFSIVA

SEQ ID NO: 96 - protein, 7 aa, synthetic construct
ITSGGNT

SEQ ID NO: 97 - protein, 16 aa, synthetic construct
NADPGVVAGPYAGMDF

SEQ ID NO: 98 - protein, 5 aa, synthetic construct
FTTMA

SEQ ID NO: 99 - protein, 16 aa, synthetic construct
SITTGGSTAYTDSVKG

SEQ ID NO: 100 - protein, 9 aa, synthetic construct
GPRNVWAAA

SEQ ID NO: 101 - protein, 10 aa, synthetic construct
GPIFSFTTMA

SEQ ID NO: 102 - protein, 9 aa, synthetic construct
SITTGGSTA

SEQ ID NO: 103 - protein, 9 aa, synthetic construct
GPRNVWAAA

SEQ ID NO: 104 - protein, 7 aa, synthetic construct
GPIFSFT

SEQ ID NO: 105 - protein, 5 aa, synthetic construct
TTGGS

SEQ ID NO: 106 - protein, 9 aa, synthetic construct
GPRNVWAAA

SEQ ID NO: 107 - protein, 8 aa, synthetic construct
GPIFSFTT

SEQ ID NO: 108 - protein, 7 aa, synthetic construct
ITTGGST

SEQ ID NO: 109 - protein, 11 aa, synthetic construct
NTGPRNVWAAA

SEQ ID NO: 110 - protein, 232 aa, synthetic construct
EPKSCDKTHTCPPCPAPELLGGPSVFLFPPKPKDTLMISRTPEVTCVVVDVSHEDPEVKFNWYVDGVEVHNAKTKPREEQYNSTYRVVSVLTVLHQDWLNGKEYKCKVSNKALPAPIEKTISKAKGQPREPQVYTLPPSRDELTKNQVSLTCLVKGFYPSDIAVEWESNGQPENNYKTTPPVLDSDGSFFLYSKLTVDKSRWQQGNVFSCSVMHEALHNHYTQKSLSLSPGK

SEQ ID NO: 111 - DNA, 29 bp, synthetic construct
  source 1..29: mol_type = other DNA
cccaccggtcaggtgcagctgcaggagtc

SEQ ID NO: 112 - DNA, 28 bp, synthetic construct
  source 1..28: mol_type = other DNA
cccggatcctgaggagacggtgacctgg

SEQ ID NO: 113 - protein, 232 aa, synthetic construct
EPKSSDKTHTCPPCPAPELLGGPSVFLFPPKPKDTLMISRTPEVTCVVVDVSHEDPEVKFNWYVDGVEVHNAKTKPREEQYNSTYRVVSVLTVLHQDWLNGKEYKCKVSNKALPAPIEKTISKAKGQPREPQVYTLPPSRDELTKNQVSLTCLVKGFYPSDIAVEWESNGQPENNYKTTPPVLDSDGSFFLYSKLTVDKSRWQQGNVFSCSVMHEALHNHYTQKSLSLSPGK